European Patent Application EP 4 303 310 A1, published January 10, 2024. Title: Ｃａｓ３タンパク質を製造する方法. Applicant: C4U Corporation The University of Tokyo RIKEN. The sequence listing filed with the application follows.

SEQUENCE LISTING (24 sequences)

SEQ ID NO: 1 - DNA, 2667 bp, Escherichia coli
  CDS (1)..(2667): EcoCas3
atggaaccttttaaatatatatgccattactggggaaaatcctcaaaaagcttgacgaaaggaaatgatattcatctgttaatttatcattgccttgatgttgctgctgttgcagattgctggtgggatcaatcagtcgtactgcaaaatactttttgccgaaatgaaatgctatcaaaacagagggtgaaggcctggctgttatttttcattgctcttcatgatattggaaagtttgatatacgattccaatataaatcagcagaaagttggctgaaattaaatcctgcaacgccatcacttaatggtccatcaacacaaatgtgccgtaaatttaatcatggtgcagccggtctgtattggtttaaccaggattcactttcagagcaatctctcggggattttttcagtttttttgatgccgctcctcatccttatgagtcctggtttccatgggtagaggccgttacaggacatcatggttttatattacattcccaggatcaagataagtcgcgttgggaaatgccagcttctctggcatcttatgctgcgcaagataaacaggctcgtgaggagtggatatctgtactggaagcattatttttaacgccagcggggttatctataaacgatataccacctgattgttcatcactgttagcaggtttttgctcgcttgctgactggttaggctcctggactacaacgaatacctttctgtttaatgaggatgcgccttccgacataaatgctctgagaacgtatttccaggaccgacagcaggatgcgagccgggtattggagttgagtggacttgtatcaaataagcgatgttatgaaggtgttcatgcactactggacaatggctatcaacccagacaattacaggtgttagttgatgctcttccagtagctcccgggctgacggtaatagaggcacctacaggctccggtaaaacggaaacagcgctggcctatgcttggaaacttattgatcaacaaattgcggatagtgttatttttgccctcccaacacaagctaccgcgaatgctatgcttacgagaatggaagcgagcgcgagccacttattttcatccccaaatcttattcttgctcatggcaattcacggtttaaccacctctttcaatcaataaaatcacgcgcgattactgaacaggggcaagaagaagcgtgggttcagtgttgtcagtggttgtcacaaagcaataagaaagtgtttcttgggcaaatcggcgtttgcacgattgatcaggtgttgatatcggtattgccagttaaacaccgctttatccgtggtttgggaattggtcgaagtgttttaattgttgatgaagttcatgcttacgacacctatatgaacggcttgctggaggcagtgctcaaggctcaggctgatgtgggagggagtgttattcttctttccgcaaccctaccaatgaaacaaaaacagaaacttctggatacttatggtctgcatacagatccagtggaaaataactccgcatatccactcattaactggcgaggtgtgaatggtgcgcaacgttttgatctgctagctcatccagaacaactcccgccccgcttttcgattcagccagaacctatttgtttagctgacatgttacctgaccttacgatgttagagcgaatgatcgcagcggcaaacgcgggtgcacaggtctgtcttatttgcaatttggttgacgttgcacaagtatgctaccaacggctaaaggagctaaataacacgcaagtagatatagatttgtttcatgcgcgctttacgctgaacgatcgtcgtgaaaaagagaatcgagttattagcaatttcggcaaaaatgggaagcgaaatgttggacggatacttgtcgcaacccaggtcgtggaacaatcactcgacgttgattttgattggttaattactcagcattgtcctgcagatttgcttttccaacgattgggccgtttacatcgccatcatcgcaaatatcgtcccgctggttttgagattcctgttgccaccattttgctgcctgatggcgagggttacggacgacatgagcatatttatagcaacgttagagtcatgtggcggacgcagcaacatattgaggagcttaatggagcatccttatttttccctgatgcttaccggcaatggctggatagcatttacgatgatgcggaaatggatgagccagaatgggtcggcaatggcatggataaatttgaaagcgccgagtgtgaaaaaaggttcaaggctcgcaaggtcctgcagtgggctgaagaatatagcttgcaggataacgatgaaaccattcttgcggtaacgagggatggggaaatgagcctgccattattgccttatgtacaaacgtcttcaggtaaacaactgctcgatggccaggtctacgaggacctaagtcatgaacagcagtatgaggcgcttgcacttaatcgcgtcaatgtacccttcacctggaaacgtagtttttctgaagtagtagatgaagatgggttactttggctggaagggaaacagaatctggatggatgggtctggcagggtaacagtattgttattacctatacaggggatgaagggatgaccagagtcatccctgcaaatcccaaataa

SEQ ID NO: 2 - protein, 888 aa, Escherichia coli
MEPFKYICHYWGKSSKSLTKGNDIHLLIYHCLDVAAVADCWWDQSVVLQNTFCRNEMLSKQRVKAWLLFFIALHDIGKFDIRFQYKSAESWLKLNPATPSLNGPSTQMCRKFNHGAAGLYWFNQDSLSEQSLGDFFSFFDAAPHPYESWFPWVEAVTGHHGFILHSQDQDKSRWEMPASLASYAAQDKQAREEWISVLEALFLTPAGLSINDIPPDCSSLLAGFCSLADWLGSWTTTNTFLFNEDAPSDINALRTYFQDRQQDASRVLELSGLVSNKRCYEGVHALLDNGYQPRQLQVLVDALPVAPGLTVIEAPTGSGKTETALAYAWKLIDQQIADSVIFALPTQATANAMLTRMEASASHLFSSPNLILAHGNSRFNHLFQSIKSRAITEQGQEEAWVQCCQWLSQSNKKVFLGQIGVCTIDQVLISVLPVKHRFIRGLGIGRSVLIVDEVHAYDTYMNGLLEAVLKAQADVGGSVILLSATLPMKQKQKLLDTYGLHTDPVENNSAYPLINWRGVNGAQRFDLLAHPEQLPPRFSIQPEPICLADMLPDLTMLERMIAAANAGAQVCLICNLVDVAQVCYQRLKELNNTQVDIDLFHARFTLNDRREKENRVISNFGKNGKRNVGRILVATQVVEQSLDVDFDWLITQHCPADLLFQRLGRLHRHHRKYRPAGFEIPVATILLPDGEGYGRHEHIYSNVRVMWRTQQHIEELNGASLFFPDAYRQWLDSIYDDAEMDEPEWVGNGMDKFESAECEKRFKARKVLQWAEEYSLQDNDETILAVTRDGEMSLPLLPYVQTSSGKQLLDGQVYEDLSHEQQYEALALNRVNVPFTWKRSFSEVVDEDGLLWLEGKQNLDGWVWQGNSIVITYTGDEGMTRVIPANPK

SEQ ID NO: 3 - protein, 7 aa, Artificial Sequence
  NLS
PKKKRKV

SEQ ID NO: 4 - protein, 18 aa, Artificial Sequence
  NLS
KRTADGSEFESPKKKRKV

SEQ ID NO: 5 - protein, 21 aa, Artificial Sequence
  HN tag
HHHHHHHHGSHNHNHNHNHNH

SEQ ID NO: 6 - DNA, 7554 bp, Artificial Sequence
  EcoCas3 plasmid
  CDS (4059)..(6908)
gacgcgccctgtagcggcgcattaagcgcggcgggtgtggtggttacgcgcagcgtgaccgctacacttgccagcgccctagcgcccgctcctttcgctttcttcccttcctttctcgccacgttcgccggctttccccgtcaagctctaaatcgggggctccctttagggttccgatttagtgctttacggcacctcgaccccaaaaaacttgattagggtgatggttcacgtagtgggccatcgccctgatagacggtttttcgccctttgacgttggagtccacgttctttaatagtggactcttgttccaaactggaacaacactcaaccctatctcggtctattcttttgatttataagggattttgccgatttcggcctattggttaaaaaatgagctgatttaacaaaaatttaacgcgaattttaacaaaatattaacgtttacaatttcaggtggcacttttcggggaaatgtgcgcggaacccctatttgtttatttttctaaatacattcaaatatgtatccgctcatgagacaataaccctgataaatgcttcaataatattgaaaaaggaagagtatgagtattcaacatttccgtgtcgcccttattcccttttttgcggcattttgccttcctgtttttgctcacccagaaacgctggtgaaagtaaaagatgctgaagatcagttgggtgcacgagtgggttacatcgaactggatctcaacagcggtaagatccttgagagttttcgccccgaagaacgttttccaatgatgagcacttttaaagttctgctatgtggcgcggtattatcccgtattgacgccgggcaagagcaactcggtcgccgcatacactattctcagaatgacttggttgagtactcaccagtcacagaaaagcatcttacggatggcatgacagtaagagaattatgcagtgctgccataaccatgagtgataacactgcggccaacttacttctgacaacgatcggaggaccgaaggagctaaccgcttttttgcacaacatgggggatcatgtaactcgccttgatcgttgggaaccggagctgaatgaagccataccaaacgacgagcgtgacaccacgatgcctgtagcaatggcaacaacgttgcgcaaactattaactggcgaactacttactctagcttcccggcaacaattaatagactggatggaggcggataaagttgcaggaccacttctgcgctcggcccttccggctggctggtttattgctgataaatctggagccggtgagcgtgggtctcgcggtatcattgcagcactggggccagatggtaagccctcccgtatcgtagttatctacacgacggggagtcaggcaactatggatgaacgaaatagacagatcgctgagataggtgcctcactgattaagcattggtaactgtcagaccaagtttactcatatatactttagattgatttaaaacttcatttttaatttaaaaggatctaggtgaagatcctttttgataatctcatgaccaaaatcccttaacgtgagttttcgttccactgagcgtcagaccccgtagaaaagatcaaaggatcttcttgagatcctttttttctgcgcgtaatctgctgcttgcaaacaaaaaaaccaccgctaccagcggtggtttgtttgccggatcaagagctaccaactctttttccgaaggtaactggcttcagcagagcgcagataccaaatactgtccttctagtgtagccgtagttaggccaccacttcaagaactctgtagcaccgcctacatacctcgctctgctaatcctgttaccagtggctgctgccagtggcgataagtcgtgtcttaccgggttggactcaagacgatagttaccggataaggcgcagcggtcgggctgaacggggggttcgtgcacacagcccagcttggagcgaacgacctacaccgaactgagatacctacagcgtgagcattgagaaagcgccacgcttcccgaagggagaaaggcggacaggtatccggtaagcggcagggtcggaacaggagagcgcacgagggagcttccagggggaaacgcctggtatctttatagtcctgtcgggtttcgccacctctgacttgagcgtcgatttttgtgatgctcgtcaggggggcggagcctatggaaaaacgccagcaacgcggcctttttacggttcctggccttttgctggccttttgctcacatgttctttcctgcgttatcccctgattctgtggataaccgtattaccgcctttgagtgagctgataccgctcgccgcagccgaacgaccgagcgcagcgagtcagtgagcgaggaagcggaagagcgcctgatgcggtattttctccttacgcatctgtgcggtatttcacaccgcagaccagccgcgtaacctggcaaaatcggttacggttgagtaataaatggatgccctgcgtaagcgggtgtgggcggacaataaagtcttaaactgaacaaaatagatctaaactatgacaataaagtcttaaactagacagaatagttgtaaactgaaatcagtccagttatgctgtgaaaaagcatactggacttttgttatggctaaagcaaactcttcattttctgaagtgcaaattgcccgtcgtattaaagaggggcgtggccaagggcatggtaaagactatattcgcggcgttgtgacaatttaccgaacaactccgcggccgggaagccgatctcggcttgaacgaattgttaggtggcggtacttgggtcgatatcaaagtgcatcacttcttcccgtatgcccaactttgtatagagagccactgcgggatcgtcaccgtaatctgcttgcacgtagatcacataagcaccaagcgcgttggcctcatgcttgaggagattgatgagcgcggtggcaatgccctgcctccggtgctcgccggagactgcgagatcatagatatagatctcactacgcggctgctcaaacctgggcagaacgtaagccgcgagagcgccaacaaccgcttcttggtcgaaggcagcaagcgcgatgaatgtcttactacggagcaagttcccgaggtaatcggagtccggctgatgttgggagtaggtggctacgtctccgaactcacgaccgaaaagatcaagagcagcccgcatggatttgacttggtcagggccgagcctacatgtgcgaatgatgcccatacttgagccacctaactttgttttagggcgactgccctgctgcgtaacatcgttgctgctgcgtaacatcgttgctgctccataacatcaaacatcgacccacggcgtaacgcgcttgctgcttggatgcccgaggcatagactgtacaaaaaaacagtcataacaagccatgaaaaccgccactgcgccgttaccaccgctgcgttcggtcaaggttctggaccagttgcgtgagcgcatacgctacttgcattacagtttacgaaccgaacaggcttatgtcaactgggttcgtgccttcatccgtttccacggtgtgcgtcacccggcaaccttgggcagcagcgaagtcgaggcatttctgtcctggctggcgaacgagcgcaaggtttcggtctccacgcatcgtcaggcattggcggccttgctgttcttctacggcaaggtgctgtgcacggatctgccctggcttcaggagatcggaagacctcggccgtcgcggcgcttgccggtggtgctgaccccggatgaagtggttcgcatcctcggttttctggaaggcgagcatcgtttgttcgcccaggactctagctatagttctagtggttggctacgtatactccggaatattaatagatcatggagataattaaaatgataaccatctcgcaaataaataagtattttactgttttcgtaacagttttgtaataaaaaaacctataaatattccggattattcataccgtcccaccatcgggcgcggatctaactcctaaaaaaccgccaccatgcatcatcaccatcaccaccatcacggttctcataaccataaccacaaccataaccacaaccacggtaccggttctgagaatctgtacttccaaggtggatcccccaagaagaagcggaaggtcggatccgaaccttttaaatatatatgccattactggggaaaatcctcaaaaagcttgacgaaaggaaatgatattcatctgttaatttatcattgccttgatgttgctgctgttgcagattgctggtgggatcaatcagtcgtactgcaaaatactttttgccgaaatgaaatgctatcaaaacagagggtgaaggcctggctgttatttttcattgctcttcatgatattggaaagtttgatatacgattccaatataaatcagcagaaagttggctgaaattaaatcctgcaacgccatcacttaatggtccatcaacacaaatgtgccgtaaatttaatcatggtgcagccggtctgtattggtttaaccaggattcactttcagagcaatctctcggggattttttcagtttttttgatgccgctcctcatccttatgagtcctggtttccatgggtagaggccgttacaggacatcatggttttatattacattcccaggatcaagataagtcgcgttgggaaatgccagcttctctggcatcttatgctgcgcaagataaacaggctcgtgaggagtggatatctgtactggaagcattatttttaacgccagcggggttatctataaacgatataccacctgattgttcatcactgttagcaggtttttgctcgcttgctgactggttaggctcctggactacaacgaatacctttctgtttaatgaggatgcgccttccgacataaatgctctgagaacgtatttccaggaccgacagcaggatgcgagccgggtattggagttgagtggacttgtatcaaataagcgatgttatgaaggtgttcatgcactactggacaatggctatcaacccagacaattacaggtgttagttgatgctcttccagtagctcccgggctgacggtaatagaggcacctacaggctccggtaaaacggaaacagcgctggcctatgcttggaaacttattgatcaacaaattgcggatagtgttatttttgccctcccaacacaagctaccgcgaatgctatgcttacgagaatggaagcgagcgcgagccacttattttcatccccaaatcttattcttgctcatggcaattcacggtttaaccacctctttcaatcaataaaatcacgcgcgattactgaacaggggcaagaagaagcgtgggttcagtgttgtcagtggttgtcacaaagcaataagaaagtgtttcttgggcaaatcggcgtttgcacgattgatcaggtgttgatatcggtattgccagttaaacaccgctttatccgtggtttgggaattggtcgaagtgttttaattgttgatgaagttcatgcttacgacacctatatgaacggcttgctggaggcagtgctcaaggctcaggctgatgtgggagggagtgttattcttctttccgcaaccctaccaatgaaacaaaaacagaaacttctggatacttatggtctgcatacagatccagtggaaaataactccgcatatccactcattaactggcgaggtgtgaatggtgcgcaacgttttgatctgctagctcatccagaacaactcccgccccgcttttcgattcagccagaacctatttgtttagctgacatgttacctgaccttacgatgttagagcgaatgatcgcagcggcaaacgcgggtgcacaggtctgtcttatttgcaatttggttgacgttgcacaagtatgctaccaacggctaaaggagctaaataacacgcaagtagatatagatttgtttcatgcgcgctttacgctgaacgatcgtcgtgaaaaagagaatcgagttattagcaatttcggcaaaaatgggaagcgaaatgttggacggatacttgtcgcaacccaggtcgtggaacaatcactcgacgttgattttgattggttaattactcagcattgtcctgcagatttgcttttccaacgattgggccgtttacatcgccatcatcgcaaatatcgtcccgctggttttgagattcctgttgccaccattttgctgcctgatggcgagggttacggacgacatgagcatatttatagcaacgttagagtcatgtggcggacgcagcaacatattgaggagcttaatggagcatccttatttttccctgatgcttaccggcaatggctggatagcatttacgatgatgcggaaatggatgagccagaatgggtcggcaatggcatggataaatttgaaagcgccgagtgtgaaaaaaggttcaaggctcgcaaggtcctgcagtgggctgaagaatatagcttgcaggataacgatgaaaccattcttgcggtaacgagggatggggaaatgagcctgccattattgccttatgtacaaacgtcttcaggtaaacaactgctcgatggccaggtctacgaggacctaagtcatgaacagcagtatgaggcgcttgcacttaatcgcgtcaatgtacccttcacctggaaacgtagtttttctgaagtagtagatgaagatgggttactttggctggaagggaaacagaatctggatggatgggtctggcagggtaacagtattgttattacctatacaggggatgaagggatgaccagagtcatccctgcaaatcccaaaaagagaacagccgatggcagcgagttcgagagccccaagaagaagcggaaggtctaactcgagaagcttgtcgagaagtactagaggatcataatcagccataccacatttgtagaggttttacttgctttaaaaaacctcccacacctccccctgaacctgaaacataaaatgaatgcaattgttgttgttaacttgtttattgcagcttataatggttacaaataaagcaatagcatcacaaatttcacaaataaagcatttttttcactgcattctagttgtggtttgtccaaactcatcaatgtatcttatcatgtctggatctgatcactgcttgagcctaggagatccgaaccagataagtgaaatctagttccaaactattttgtcatttttaattttcgtattagcttacgacgctacacccagttcccatctattttgtcactcttccctaaataatccttaaaaactccatttccacccctcccagttcccaactattttgtccgcccacagcggggcatttttcttcctgttatgtttttaatcaaacatcctgccaactccatgtgacaaaccgtcatcttcggctactttttctctgtcacagaatgaaaatttttctgtcatctcttcgttattaatgtttgtaattgactgaatatcaacgcttatttgcagcctgaatggcgaatgg

SEQ ID NO: 7 - protein, 949 aa, Artificial Sequence
  Synthetic Construct
MHHHHHHHHGSHNHNHNHNHNHGTGSENLYFQGGSPKKKRKVGSEPFKYICHYWGKSSKSLTKGNDIHLLIYHCLDVAAVADCWWDQSVVLQNTFCRNEMLSKQRVKAWLLFFIALHDIGKFDIRFQYKSAESWLKLNPATPSLNGPSTQMCRKFNHGAAGLYWFNQDSLSEQSLGDFFSFFDAAPHPYESWFPWVEAVTGHHGFILHSQDQDKSRWEMPASLASYAAQDKQAREEWISVLEALFLTPAGLSINDIPPDCSSLLAGFCSLADWLGSWTTTNTFLFNEDAPSDINALRTYFQDRQQDASRVLELSGLVSNKRCYEGVHALLDNGYQPRQLQVLVDALPVAPGLTVIEAPTGSGKTETALAYAWKLIDQQIADSVIFALPTQATANAMLTRMEASASHLFSSPNLILAHGNSRFNHLFQSIKSRAITEQGQEEAWVQCCQWLSQSNKKVFLGQIGVCTIDQVLISVLPVKHRFIRGLGIGRSVLIVDEVHAYDTYMNGLLEAVLKAQADVGGSVILLSATLPMKQKQKLLDTYGLHTDPVENNSAYPLINWRGVNGAQRFDLLAHPEQLPPRFSIQPEPICLADMLPDLTMLERMIAAANAGAQVCLICNLVDVAQVCYQRLKELNNTQVDIDLFHARFTLNDRREKENRVISNFGKNGKRNVGRILVATQVVEQSLDVDFDWLITQHCPADLLFQRLGRLHRHHRKYRPAGFEIPVATILLPDGEGYGRHEHIYSNVRVMWRTQQHIEELNGASLFFPDAYRQWLDSIYDDAEMDEPEWVGNGMDKFESAECEKRFKARKVLQWAEEYSLQDNDETILAVTRDGEMSLPLLPYVQTSSGKQLLDGQVYEDLSHEQQYEALALNRVNVPFTWKRSFSEVVDEDGLLWLEGKQNLDGWVWQGNSIVITYTGDEGMTRVIPANPKKRTADGSEFESPKKKRKV

SEQ ID NO: 8 - DNA, 8274 bp, Artificial Sequence
  EGFP-EcoCas3 plasmid
  CDS (4059)..(7628)
gacgcgccctgtagcggcgcattaagcgcggcgggtgtggtggttacgcgcagcgtgaccgctacacttgccagcgccctagcgcccgctcctttcgctttcttcccttcctttctcgccacgttcgccggctttccccgtcaagctctaaatcgggggctccctttagggttccgatttagtgctttacggcacctcgaccccaaaaaacttgattagggtgatggttcacgtagtgggccatcgccctgatagacggtttttcgccctttgacgttggagtccacgttctttaatagtggactcttgttccaaactggaacaacactcaaccctatctcggtctattcttttgatttataagggattttgccgatttcggcctattggttaaaaaatgagctgatttaacaaaaatttaacgcgaattttaacaaaatattaacgtttacaatttcaggtggcacttttcggggaaatgtgcgcggaacccctatttgtttatttttctaaatacattcaaatatgtatccgctcatgagacaataaccctgataaatgcttcaataatattgaaaaaggaagagtatgagtattcaacatttccgtgtcgcccttattcccttttttgcggcattttgccttcctgtttttgctcacccagaaacgctggtgaaagtaaaagatgctgaagatcagttgggtgcacgagtgggttacatcgaactggatctcaacagcggtaagatccttgagagttttcgccccgaagaacgttttccaatgatgagcacttttaaagttctgctatgtggcgcggtattatcccgtattgacgccgggcaagagcaactcggtcgccgcatacactattctcagaatgacttggttgagtactcaccagtcacagaaaagcatcttacggatggcatgacagtaagagaattatgcagtgctgccataaccatgagtgataacactgcggccaacttacttctgacaacgatcggaggaccgaaggagctaaccgcttttttgcacaacatgggggatcatgtaactcgccttgatcgttgggaaccggagctgaatgaagccataccaaacgacgagcgtgacaccacgatgcctgtagcaatggcaacaacgttgcgcaaactattaactggcgaactacttactctagcttcccggcaacaattaatagactggatggaggcggataaagttgcaggaccacttctgcgctcggcccttccggctggctggtttattgctgataaatctggagccggtgagcgtgggtctcgcggtatcattgcagcactggggccagatggtaagccctcccgtatcgtagttatctacacgacggggagtcaggcaactatggatgaacgaaatagacagatcgctgagataggtgcctcactgattaagcattggtaactgtcagaccaagtttactcatatatactttagattgatttaaaacttcatttttaatttaaaaggatctaggtgaagatcctttttgataatctcatgaccaaaatcccttaacgtgagttttcgttccactgagcgtcagaccccgtagaaaagatcaaaggatcttcttgagatcctttttttctgcgcgtaatctgctgcttgcaaacaaaaaaaccaccgctaccagcggtggtttgtttgccggatcaagagctaccaactctttttccgaaggtaactggcttcagcagagcgcagataccaaatactgtccttctagtgtagccgtagttaggccaccacttcaagaactctgtagcaccgcctacatacctcgctctgctaatcctgttaccagtggctgctgccagtggcgataagtcgtgtcttaccgggttggactcaagacgatagttaccggataaggcgcagcggtcgggctgaacggggggttcgtgcacacagcccagcttggagcgaacgacctacaccgaactgagatacctacagcgtgagcattgagaaagcgccacgcttcccgaagggagaaaggcggacaggtatccggtaagcggcagggtcggaacaggagagcgcacgagggagcttccagggggaaacgcctggtatctttatagtcctgtcgggtttcgccacctctgacttgagcgtcgatttttgtgatgctcgtcaggggggcggagcctatggaaaaacgccagcaacgcggcctttttacggttcctggccttttgctggccttttgctcacatgttctttcctgcgttatcccctgattctgtggataaccgtattaccgcctttgagtgagctgataccgctcgccgcagccgaacgaccgagcgcagcgagtcagtgagcgaggaagcggaagagcgcctgatgcggtattttctccttacgcatctgtgcggtatttcacaccgcagaccagccgcgtaacctggcaaaatcggttacggttgagtaataaatggatgccctgcgtaagcgggtgtgggcggacaataaagtcttaaactgaacaaaatagatctaaactatgacaataaagtcttaaactagacagaatagttgtaaactgaaatcagtccagttatgctgtgaaaaagcatactggacttttgttatggctaaagcaaactcttcattttctgaagtgcaaattgcccgtcgtattaaagaggggcgtggccaagggcatggtaaagactatattcgcggcgttgtgacaatttaccgaacaactccgcggccgggaagccgatctcggcttgaacgaattgttaggtggcggtacttgggtcgatatcaaagtgcatcacttcttcccgtatgcccaactttgtatagagagccactgcgggatcgtcaccgtaatctgcttgcacgtagatcacataagcaccaagcgcgttggcctcatgcttgaggagattgatgagcgcggtggcaatgccctgcctccggtgctcgccggagactgcgagatcatagatatagatctcactacgcggctgctcaaacctgggcagaacgtaagccgcgagagcgccaacaaccgcttcttggtcgaaggcagcaagcgcgatgaatgtcttactacggagcaagttcccgaggtaatcggagtccggctgatgttgggagtaggtggctacgtctccgaactcacgaccgaaaagatcaagagcagcccgcatggatttgacttggtcagggccgagcctacatgtgcgaatgatgcccatacttgagccacctaactttgttttagggcgactgccctgctgcgtaacatcgttgctgctgcgtaacatcgttgctgctccataacatcaaacatcgacccacggcgtaacgcgcttgctgcttggatgcccgaggcatagactgtacaaaaaaacagtcataacaagccatgaaaaccgccactgcgccgttaccaccgctgcgttcggtcaaggttctggaccagttgcgtgagcgcatacgctacttgcattacagtttacgaaccgaacaggcttatgtcaactgggttcgtgccttcatccgtttccacggtgtgcgtcacccggcaaccttgggcagcagcgaagtcgaggcatttctgtcctggctggcgaacgagcgcaaggtttcggtctccacgcatcgtcaggcattggcggccttgctgttcttctacggcaaggtgctgtgcacggatctgccctggcttcaggagatcggaagacctcggccgtcgcggcgcttgccggtggtgctgaccccggatgaagtggttcgcatcctcggttttctggaaggcgagcatcgtttgttcgcccaggactctagctatagttctagtggttggctacgtatactccggaatattaatagatcatggagataattaaaatgataaccatctcgcaaataaataagtattttactgttttcgtaacagttttgtaataaaaaaacctataaatattccggattattcataccgtcccaccatcgggcgcggatctaactcctaaaaaaccgccaccatgcatcatcaccatcaccaccatcacggttctcataaccataaccacaaccataaccacaaccacggtaccgtgagcaagggcgaggagctgttcaccggggtggtgcccatcctggtcgagctggacggcgacgtaaacggccacaagttcagcgtgtccggcgagggcgagggcgatgccacctacggcaagctgaccctgaagttcatctgcaccaccggcaagctgcccgtgccctggcccaccctcgtgaccaccctgacctacggcgtgcagtgcttcagccgctaccccgaccacatgaagcagcacgacttcttcaagtccgccatgcccgaaggctacgtccaggagcgcaccatcttcttcaaggacgacggcaactacaagacccgcgccgaggtgaagttcgagggcgacaccctggtgaaccgcatcgagctgaagggcatcgacttcaaggaggacggcaacatcctggggcacaagctggagtacaactacaacagccacaacgtctatatcatggccgacaagcagaagaacggcatcaaggtgaacttcaagatccgccacaacatcgaggacggcagcgtgcagctcgccgaccactaccagcagaacacccccatcggcgacggccccgtgctgctgcccgacaaccactacctgagcacccagtccaaactgagcaaagaccccaacgagaagcgcgatcacatggtcctgctggagttcgtgaccgccgccgggatcactctcggcatggacgagctgtacaagggtaccggttctgagaatctgtacttccaaggtggatcccccaagaagaagcggaaggtcggatccgaaccttttaaatatatatgccattactggggaaaatcctcaaaaagcttgacgaaaggaaatgatattcatctgttaatttatcattgccttgatgttgctgctgttgcagattgctggtgggatcaatcagtcgtactgcaaaatactttttgccgaaatgaaatgctatcaaaacagagggtgaaggcctggctgttatttttcattgctcttcatgatattggaaagtttgatatacgattccaatataaatcagcagaaagttggctgaaattaaatcctgcaacgccatcacttaatggtccatcaacacaaatgtgccgtaaatttaatcatggtgcagccggtctgtattggtttaaccaggattcactttcagagcaatctctcggggattttttcagtttttttgatgccgctcctcatccttatgagtcctggtttccatgggtagaggccgttacaggacatcatggttttatattacattcccaggatcaagataagtcgcgttgggaaatgccagcttctctggcatcttatgctgcgcaagataaacaggctcgtgaggagtggatatctgtactggaagcattatttttaacgccagcggggttatctataaacgatataccacctgattgttcatcactgttagcaggtttttgctcgcttgctgactggttaggctcctggactacaacgaatacctttctgtttaatgaggatgcgccttccgacataaatgctctgagaacgtatttccaggaccgacagcaggatgcgagccgggtattggagttgagtggacttgtatcaaataagcgatgttatgaaggtgttcatgcactactggacaatggctatcaacccagacaattacaggtgttagttgatgctcttccagtagctcccgggctgacggtaatagaggcacctacaggctccggtaaaacggaaacagcgctggcctatgcttggaaacttattgatcaacaaattgcggatagtgttatttttgccctcccaacacaagctaccgcgaatgctatgcttacgagaatggaagcgagcgcgagccacttattttcatccccaaatcttattcttgctcatggcaattcacggtttaaccacctctttcaatcaataaaatcacgcgcgattactgaacaggggcaagaagaagcgtgggttcagtgttgtcagtggttgtcacaaagcaataagaaagtgtttcttgggcaaatcggcgtttgcacgattgatcaggtgttgatatcggtattgccagttaaacaccgctttatccgtggtttgggaattggtcgaagtgttttaattgttgatgaagttcatgcttacgacacctatatgaacggcttgctggaggcagtgctcaaggctcaggctgatgtgggagggagtgttattcttctttccgcaaccctaccaatgaaacaaaaacagaaacttctggatacttatggtctgcatacagatccagtggaaaataactccgcatatccactcattaactggcgaggtgtgaatggtgcgcaacgttttgatctgctagctcatccagaacaactcccgccccgcttttcgattcagccagaacctatttgtttagctgacatgttacctgaccttacgatgttagagcgaatgatcgcagcggcaaacgcgggtgcacaggtctgtcttatttgcaatttggttgacgttgcacaagtatgctaccaacggctaaaggagctaaataacacgcaagtagatatagatttgtttcatgcgcgctttacgctgaacgatcgtcgtgaaaaagagaatcgagttattagcaatttcggcaaaaatgggaagcgaaatgttggacggatacttgtcgcaacccaggtcgtggaacaatcactcgacgttgattttgattggttaattactcagcattgtcctgcagatttgcttttccaacgattgggccgtttacatcgccatcatcgcaaatatcgtcccgctggttttgagattcctgttgccaccattttgctgcctgatggcgagggttacggacgacatgagcatatttatagcaacgttagagtcatgtggcggacgcagcaacatattgaggagcttaatggagcatccttatttttccctgatgcttaccggcaatggctggatagcatttacgatgatgcggaaatggatgagccagaatgggtcggcaatggcatggataaatttgaaagcgccgagtgtgaaaaaaggttcaaggctcgcaaggtcctgcagtgggctgaagaatatagcttgcaggataacgatgaaaccattcttgcggtaacgagggatggggaaatgagcctgccattattgccttatgtacaaacgtcttcaggtaaacaactgctcgatggccaggtctacgaggacctaagtcatgaacagcagtatgaggcgcttgcacttaatcgcgtcaatgtacccttcacctggaaacgtagtttttctgaagtagtagatgaagatgggttactttggctggaagggaaacagaatctggatggatgggtctggcagggtaacagtattgttattacctatacaggggatgaagggatgaccagagtcatccctgcaaatcccaaaaagagaacagccgatggcagcgagttcgagagccccaagaagaagcggaaggtctaactcgagaagcttgtcgagaagtactagaggatcataatcagccataccacatttgtagaggttttacttgctttaaaaaacctcccacacctccccctgaacctgaaacataaaatgaatgcaattgttgttgttaacttgtttattgcagcttataatggttacaaataaagcaatagcatcacaaatttcacaaataaagcatttttttcactgcattctagttgtggtttgtccaaactcatcaatgtatcttatcatgtctggatctgatcactgcttgagcctaggagatccgaaccagataagtgaaatctagttccaaactattttgtcatttttaattttcgtattagcttacgacgctacacccagttcccatctattttgtcactcttccctaaataatccttaaaaactccatttccacccctcccagttcccaactattttgtccgcccacagcggggcatttttcttcctgttatgtttttaatcaaacatcctgccaactccatgtgacaaaccgtcatcttcggctactttttctctgtcacagaatgaaaatttttctgtcatctcttcgttattaatgtttgtaattgactgaatatcaacgcttatttgcagcctgaatggcgaatgg

SEQ ID NO: 9 - protein, 1189 aa, Artificial Sequence
  Synthetic Construct
MHHHHHHHHGSHNHNHNHNHNHGTVSKGEELFTGVVPILVELDGDVNGHKFSVSGEGEGDATYGKLTLKFICTTGKLPVPWPTLVTTLTYGVQCFSRYPDHMKQHDFFKSAMPEGYVQERTIFFKDDGNYKTRAEVKFEGDTLVNRIELKGIDFKEDGNILGHKLEYNYNSHNVYIMADKQKNGIKVNFKIRHNIEDGSVQLADHYQQNTPIGDGPVLLPDNHYLSTQSKLSKDPNEKRDHMVLLEFVTAAGITLGMDELYKGTGSENLYFQGGSPKKKRKVGSEPFKYICHYWGKSSKSLTKGNDIHLLIYHCLDVAAVADCWWDQSVVLQNTFCRNEMLSKQRVKAWLLFFIALHDIGKFDIRFQYKSAESWLKLNPATPSLNGPSTQMCRKFNHGAAGLYWFNQDSLSEQSLGDFFSFFDAAPHPYESWFPWVEAVTGHHGFILHSQDQDKSRWEMPASLASYAAQDKQAREEWISVLEALFLTPAGLSINDIPPDCSSLLAGFCSLADWLGSWTTTNTFLFNEDAPSDINALRTYFQDRQQDASRVLELSGLVSNKRCYEGVHALLDNGYQPRQLQVLVDALPVAPGLTVIEAPTGSGKTETALAYAWKLIDQQIADSVIFALPTQATANAMLTRMEASASHLFSSPNLILAHGNSRFNHLFQSIKSRAITEQGQEEAWVQCCQWLSQSNKKVFLGQIGVCTIDQVLISVLPVKHRFIRGLGIGRSVLIVDEVHAYDTYMNGLLEAVLKAQADVGGSVILLSATLPMKQKQKLLDTYGLHTDPVENNSAYPLINWRGVNGAQRFDLLAHPEQLPPRFSIQPEPICLADMLPDLTMLERMIAAANAGAQVCLICNLVDVAQVCYQRLKELNNTQVDIDLFHARFTLNDRREKENRVISNFGKNGKRNVGRILVATQVVEQSLDVDFDWLITQHCPADLLFQRLGRLHRHHRKYRPAGFEIPVATILLPDGEGYGRHEHIYSNVRVMWRTQQHIEELNGASLFFPDAYRQWLDSIYDDAEMDEPEWVGNGMDKFESAECEKRFKARKVLQWAEEYSLQDNDETILAVTRDGEMSLPLLPYVQTSSGKQLLDGQVYEDLSHEQQYEALALNRVNVPFTWKRSFSEVVDEDGLLWLEGKQNLDGWVWQGNSIVITYTGDEGMTRVIPANPKKRTADGSEFESPKKKRKV

SEQ ID NO: 10 - DNA, 4299 bp, Artificial Sequence
  HisTag-Cas11-bpNLS/pCDFDuet-1
  CDS (71)..(667)
ggggaattgtgagcggataacaattcccctgtagaaataattttgtttaactttaataaggagatataccatggcaagccatcatcaccatcaccatcaccatggttctctggaagttctgttccaggggcccgctgatgaaattgatgcaatggctttatatcgagcctggcaacaactggataatggatcatgtgcgcaaattagacgtgtttcagaacctgatgaattacgcgatatccctgcgttttataggctggtgcaaccttttggttgggaaaacccacgtcaccagcaggctcttttgcgcatggtgttttgcctgagcgcaggaaagaatgtcatccgacatcaggacaaaaaatcggagcaaacaacaggtatctcgttgggaagagctttagccaatagtggaagaattaacgagcgccgtatctttcaattaattcgggctgacagaacagccgatatggtccagttacgtcgattacttactcacgccgaacccgtacttgactggccattaatggccaggatgttgacctggtggggaaagcgcgaacgccagcaacttctggaagattttgtattgaccacaaacaaaaatgcgaagagaacagccgatggcagcgagttcgagagccccaagaagaagcggaaggtctaagcggccgcataatgcttaagtcgaacagaaagtaatcgtattgtacacggccgcataatcgaaattaatacgactcactataggggaattgtgagcggataacaattccccatcttagtatattagttaagtataagaaggagatatacatatggcagatctcaattggatatcggccggccacgcgatcgctgacgtcggtaccctcgagtctggtaaagaaaccgctgctgcgaaatttgaacgccagcacatggactcgtctactagcgcagcttaattaacctaggctgctgccaccgctgagcaataactagcataaccccttggggcctctaaacgggtcttgaggggttttttgctgaaacctcaggcatttgagaagcacacggtcacactgcttccggtagtcaataaaccggtaaaccagcaatagacataagcggctatttaacgaccctgccctgaaccgacgaccgggtcatcgtggccggatcttgcggcccctcggcttgaacgaattgttagacattatttgccgactaccttggtgatctcgcctttcacgtagtggacaaattcttccaactgatctgcgcgcgaggccaagcgatcttcttcttgtccaagataagcctgtctagcttcaagtatgacgggctgatactgggccggcaggcgctccattgcccagtcggcagcgacatccttcggcgcgattttgccggttactgcgctgtaccaaatgcgggacaacgtaagcactacatttcgctcatcgccagcccagtcgggcggcgagttccatagcgttaaggtttcatttagcgcctcaaatagatcctgttcaggaaccggatcaaagagttcctccgccgctggacctaccaaggcaacgctatgttctcttgcttttgtcagcaagatagccagatcaatgtcgatcgtggctggctcgaagatacctgcaagaatgtcattgcgctgccattctccaaattgcagttcgcgcttagctggataacgccacggaatgatgtcgtcgtgcacaacaatggtgacttctacagcgcggagaatctcctctctccaggggaagccgaagtttccaaaaggtcgttgatcaaagctcgccgcgttgtttcatcaagccttacggtcaccgtaaccagcaaatcaatatcactgtgtggcttcaggccgccatccactgcggagccgtacaaatgtacggccagcaacgtcggttcgagatggcgctcgatgacgccaactacctctgatagttgagtcgatacttcggcgatcaccgcttccctcatactcttcctttttcaatattattgaagcatttatcagggttattgtctcatgagcggatacatatttgaatgtatttagaaaaataaacaaatagctagctcactcggtcgctacgctccgggcgtgagactgcggcgggcgctgcggacacatacaaagttacccacagattccgtggataagcaggggactaacatgtgaggcaaaacagcagggccgcgccggtggcgtttttccataggctccgccctcctgccagagttcacataaacagacgcttttccggtgcatctgtgggagccgtgaggctcaaccatgaatctgacagtacgggcgaaacccgacaggacttaaagatccccaccgtttccggcgggtcgctccctcttgcgctctcctgttccgaccctgccgtttaccggatacctgttccgcctttctcccttacgggaagtgtggcgctttctcatagctcacacactggtatctcggctcggtgtaggtcgttcgctccaagctgggctgtaagcaagaactccccgttcagcccgactgctgcgccttatccggtaactgttcacttgagtccaacccggaaaagcacggtaaaacgccactggcagcagccattggtaactgggagttcgcagaggatttgtttagctaaacacgcggttgctcttgaagtgtgcgccaaagtccggctacactggaaggacagatttggttgctgtgctctgcgaaagccagttaccacggttaagcagttccccaactgacttaaccttcgatcaaaccacctccccaggtggttttttcgtttacagggcaaaagattacgcgcagaaaaaaaggatctcaagaagatcctttgatcttttctactgaaccgctctagatttcagtgcaatttatctcttcaaatgtagcacctgaagtcagccccatacgatataagttgtaattctcatgttagtcatgccccgcgcccaccggaaggagctgactgggttgaaggctctcaagggcatcggtcgagatcccggtgcctaatgagtgagctaacttacattaattgcgttgcgctcactgcccgctttccagtcgggaaacctgtcgtgccagctgcattaatgaatcggccaacgcgcggggagaggcggtttgcgtattgggcgccagggtggtttttcttttcaccagtgagacgggcaacagctgattgcccttcaccgcctggccctgagagagttgcagcaagcggtccacgctggtttgccccagcaggcgaaaatcctgtttgatggtggttaacggcgggatataacatgagctgtcttcggtatcgtcgtatcccactaccgagatgtccgcaccaacgcgcagcccggactcggtaatggcgcgcattgcgcccagcgccatctgatcgttggcaaccagcatcgcagtgggaacgatgccctcattcagcatttgcatggtttgttgaaaaccggacatggcactccagtcgccttcccgttccgctatcggctgaatttgattgcgagtgagatatttatgccagccagccagacgcagacgcgccgagacagaacttaatgggcccgctaacagcgcgatttgctggtgacccaatgcgaccagatgctccacgcccagtcgcgtaccgtcttcatgggagaaaataatactgttgatgggtgtctggtcagagacatcaagaaataacgccggaacattagtgcaggcagcttccacagcaatggcatcctggtcatccagcggatagttaatgatcagcccactgacgcgttgcgcgagaagattgtgcaccgccgctttacaggcttcgacgccgcttcgttctaccatcgacaccaccacgctggcacccagttgatcggcgcgagatttaatcgccgcgacaatttgcgacggcgcgtgcagggccagactggaggtggcaacgccaatcagcaacgactgtttgcccgccagttgttgtgccacgcggttgggaatgtaattcagctccgccatcgccgcttccactttttcccgcgttttcgcagaaacgtggctggcctggttcaccacgcgggaaacggtctgataagagacaccggcatactctgcgacatcgtataacgttactggtttcacattcaccaccctgaattgactctcttccgggcgctatcatgccataccgcgaaaggttttgcgccattcgatggtgtccgggatctcgacgctctcccttatgcgactcctgcattaggaaattaatacgactcactata

SEQ ID NO: 11 - protein, 198 aa, Artificial Sequence
  Synthetic Construct
MASHHHHHHHHGSLEVLFQGPADEIDAMALYRAWQQLDNGSCAQIRRVSEPDELRDIPAFYRLVQPFGWENPRHQQALLRMVFCLSAGKNVIRHQDKKSEQTTGISLGRALANSGRINERRIFQLIRADRTADMVQLRRLLTHAEPVLDWPLMARMLTWWGKRERQQLLEDFVLTTNKNAKRTADGSEFESPKKKRKV

SEQ ID NO: 12 - DNA, 8166 bp, Artificial Sequence
  (Cas8-Cas11-Cas7-bpNLS)+(Cas5-Cas6-bpNLS)/pRSFDuet-1
  CDS (71)..(1585): Cas8
ggggaattgtgagcggataacaattcccctgtagaaataattttgtttaactttaataaggagatataccatggaaatgaatttgcttattgataactggatccctgtacgcccgcgaaacggggggaaagtccaaatcataaatctgcaatcgctatactgcagtagagatcagtggcgattaagtttgccccgtgacgatatggaactggccgctttagcactgctggtttgcattgggcaaattatcgccccggcaaaagatgacgttgaatttcgacatcgcataatgaatccgctcactgaagatgagtttcaacaactcatcgcgccgtggatagatatgttctaccttaatcacgcagaacatccctttatgcagaccaaaggtgtcaaagcaaatgatgtgactccaatggaaaaactgttggctggggtaagcggcgcgacgaattgtgcatttgtcaatcaaccggggcagggtgaagcattatgtggtggatgcactgcgattgcgttattcaaccaggcgaatcaggcaccaggttttggtggtggttttaaaagcggtttacgtggaggaacacctgtaacaacgttcgtacgtgggatcgatcttcgttcaacggtgttactcaatgtcctcacattacctcgtcttcaaaaacaatttcctaatgaatcacatacggaaaaccaacctacctggattaaacctatcaagtccaatgagtctatacctgcttcgtcaattgggtttgtccgtggtctattctggcaaccagcgcatattgaattatgcgatcccattgggattggtaaatgttcttgctgtggacaggaaagcaatttgcgttataccggttttcttaaggaaaaatttacctttacagttaatgggctatggccccatccgcattccccttgtctggtaacagtcaagaaaggggaggttgaggaaaaatttcttgctttcaccacctccgcaccatcatggacacaaatcagccgagttgtggtagataagattattcaaaatgaaaatggaaatcgcgtggcggcggttgtgaatcaattcagaaatattgcgccgcaaagtcctcttgaattgattatggggggatatcgtaataatcaagcatctattcttgaacggcgtcatgatgtgttgatgtttaatcaggggtggcaacaatacggcaatgtgataaacgaaatagtgactgttggtttgggatataaaacagccttacgcaaggcgttatatacctttgcagaagggtttaaaaataaagacttcaaaggggccggagtctctgttcatgagactgcagaaaggcatttctatcgacagagtgaattattaattcccgatgtactggcgaatgttaatttttcccaggctgatgaggtaatagctgatttacgagacaaacttcatcaattgtgtgaaatgctatttaatcaatctgtagctccctatgcacatcatcctaaattaataagcacattagcgcttgcccgcgccacgctatacaaacatttacgggagttaaaaccgcaaggagggccatcaaatggctgatgaaattgatgcaatggctttatatcgagcctggcaacaactggataatggatcatgtgcgcaaattagacgtgtttcagaacctgatgaattacgcgatatccctgcgttttataggctggtgcaaccttttggttgggaaaacccacgtcaccagcaggctcttttgcgcatggtgttttgcctgagcgcaggaaagaatgtcatccgacatcaggacaaaaaatcggagcaaacaacaggtatctcgttgggaagagctttagccaatagtggaagaattaacgagcgccgtatctttcaattaattcgggctgacagaacagccgatatggtccagttacgtcgattacttactcacgccgaacccgtacttgactggccattaatggccaggatgttgacctggtggggaaagcgcgaacgccagcaacttctggaagattttgtattgaccacaaacaaaaatgcgtaaggaaacctttctatgtctaactttatcaatattcatgttctgatctctcacagcccttcatgtctgaaccgcgacgatatgaacatgcagaaagacgctattttcggcggcaaaagacgagtaagaatttcaagtcaaagccttaaacgtgcgatgcgtaaaagtggttattacgcacaaaatattggtgaatccagtctcagaaccattcatcttgcacaattacgtgatgttcttcggcaaaaacttggtgaacgttttgaccaaaaaatcatcgataagacattagcgctgctctccggtaaatcagttgatgaagccgaaaagatttctgccgatgcggttactccctgggttgtgggagaaatagcctggttctgtgagcaggttgcaaaagcagaggctgataatctggatgataaaaagctgctcaaagttcttaaggaagatattgccgccatacgtgtgaatttacagcagggtgttgatattgcgcttagtggaagaatggcaaccagcggcatgatgactgagttgggaaaagttgatggtgcaatgtccattgcgcatgcgatcactactcatcaggttgattctgatattgactggttcaccgctgtagatgatttacaggaacaaggttctgcacatctgggaactcaggaattttcatcgggtgttttttatcgttatgccaacattaacctcgctcaacttcaggaaaatttaggtggtgcctccagggagcaggctctggaaattgcaacccatgttgttcatatgctggcaacagaggtccctggagcaaaacagcgtacttatgccgcttttaaccctgcggatatggtaatggttaatttctccgatatgccactttctatggcaaatgcttttgaaaaagcggttaaagcgaaagatggctttttgcaaccgtctatacaggcgtttaatcaatattgggatcgcgttgccaatggatatggtctgaacggagctgctgcgcaattcagcttatctgatgtagacccaattactgctcaagttaaacaaatgcctactttagaacagttaaaatcctgggttcgtaataatggcgaggcgaagagaacagccgatggcagcgagttcgagagccccaagaagaagcggaaggtctgaaagcttgcggccgcataatgcttaagtcgaacagaaagtaatcgtattgtacacggccgcataatcgaaattaatacgactcactataggggaattgtgagcggataacaattccccatcttagtatattagttaagtataagaaggagatatacatatgagatcttatttgatcttgcggcttgctgggccaatgcaagcctgggggcagccgacctttgaaggaacgcgacctaccggaagatttccgacccgaagcgggttattagggctactcggggcttgtcttgggatccaacgtgatgatacttcttcattacaggcgttatcagagagtgtgcaatttgcagtgcgctgcgatgaactcattcttgacgatcgtcgtgtgtctgtaacggggttgcgtgattaccatacagtccttggagcgcgagaagattaccgtggtttgaaaagtcatgaaacgattcaaacatggcgcgaatatttatgtgatgcctcctttaccgtcgctctctggttaacaccccatgcaacgatggttatctcagaacttgaaaaagcagtattaaagcctcggtatacaccttacctggggcggagaagttgcccactaacacacccgctttttttggggacatgtcaggcatcggatcctcagaaggcgctattaaattatgagcccgttggcggcgatatatatagtgaggaatcagttacagggcatcatttaaaatttacggcgcgcgacgaaccgatgatcaccttgcctcgacaatttgcttcccgagaatggtatgtgattaaaggaggtatggatgtatctcagtaaagtcatcattgccagggcctggagcagggatctttaccaacttcaccagggattatggcatttatttccaaacagaccggatgctgctcgtgattttctttttcatgttgagaagcgaaacacaccagaaggctgtcatgttttattgcagtcagcgcaaatgcctgtttcaactgccgttgcgacagtcattaaaactaaacaggttgaatttcaacttcaggttggtgttccactctattttcggcttcgggcaaatccgatcaaaactattctcgacaatcaaaagcgcctggacagtaaagggaatattaaacgctgtcgggttccgttaataaaagaagcagaacaaatcgcgtggttgcaacgtaaattgggcaatgcggcgcgcgttgaagatgtgcatcccatatcggaacggccacagtatttttctggtgatggtaaaagtggaaagatccaaacggtttgctttgaaggtgtgctcaccatcaacgacgcgccagcgttaatagatcttgtacagcaaggtattgggccagctaaatcgatgggatgtggcttgctatctttggctccactgaagagaacagccgatggcagcgagttcgagagccccaagaagaagcggaaggtctgactcgagtctggtaaagaaaccgctgctgcgaaatttgaacgccagcacatggactcgtctactagcgcagcttaattaacctaggctgctgccaccgctgagcaataactagcataaccccttggggcctctaaacgggtcttgaggggttttttgctgaaacctcaggcatttgagaagcacacggtcacactgcttccggtagtcaataaaccggtaaaccagcaatagacataagcggctatttaacgaccctgccctgaaccgacgacaagctgacgaccgggtctccgcaagtggcacttttcggggaaatgtgcgcggaacccctatttgtttatttttctaaatacattcaaatatgtatccgctcatgaattaattcttagaaaaactcatcgagcatcaaatgaaactgcaatttattcatatcaggattatcaataccatatttttgaaaaagccgtttctgtaatgaaggagaaaactcaccgaggcagttccataggatggcaagatcctggtatcggtctgcgattccgactcgtccaacatcaatacaacctattaatttcccctcgtcaaaaataaggttatcaagtgagaaatcaccatgagtgacgactgaatccggtgagaatggcaaaagtttatgcatttctttccagacttgttcaacaggccagccattacgctcgtcatcaaaatcactcgcatcaaccaaaccgttattcattcgtgattgcgcctgagcgagacgaaatacgcggtcgctgttaaaaggacaattacaaacaggaatcgaatgcaaccggcgcaggaacactgccagcgcatcaacaatattttcacctgaatcaggatattcttctaatacctggaatgctgttttcccggggatcgcagtggtgagtaaccatgcatcatcaggagtacggataaaatgcttgatggtcggaagaggcataaattccgtcagccagtttagtctgaccatctcatctgtaacatcattggcaacgctacctttgccatgtttcagaaacaactctggcgcatcgggcttcccatacaatcgatagattgtcgcacctgattgcccgacattatcgcgagcccatttatacccatataaatcagcatccatgttggaatttaatcgcggcctagagcaagacgtttcccgttgaatatggctcatactcttcctttttcaatattattgaagcatttatcagggttattgtctcatgagcggatacatatttgaatgtatttagaaaaataaacaaataggcatgcagcgctcttccgcttcctcgctcactgactcgctacgctcggtcgttcgactgcggcgagcggtgtcagctcactcaaaagcggtaatacggttatccacagaatcaggggataaagccggaaagaacatgtgagcaaaaagcaaagcaccggaagaagccaacgccgcaggcgtttttccataggctccgcccccctgacgagcatcacaaaaatcgacgctcaagccagaggtggcgaaacccgacaggactataaagataccaggcgtttccccctggaagctccctcgtgcgctctcctgttccgaccctgccgcttaccggatacctgtccgcctttctcccttcgggaagcgtggcgctttctcatagctcacgctgttggtatctcagttcggtgtaggtcgttcgctccaagctgggctgtgtgcacgaaccccccgttcagcccgaccgctgcgccttatccggtaactatcgtcttgagtccaacccggtaagacacgacttatcgccactggcagcagccattggtaactgatttagaggactttgtcttgaagttatgcacctgttaaggctaaactgaaagaacagattttggtgagtgcggtcctccaacccacttaccttggttcaaagagttggtagctcagcgaaccttgagaaaaccaccgttggtagcggtggtttttctttatttatgagatgatgaatcaatcggtctatcaagtcaacgaacagctattccgttactctagatttcagtgcaatttatctcttcaaatgtagcacctgaagtcagccccatacgatataagttgtaattctcatgttagtcatgccccgcgcccaccggaaggagctgactgggttgaaggctctcaagggcatcggtcgagatcccggtgcctaatgagtgagctaacttacattaattgcgttgcgctcactgcccgctttccagtcgggaaacctgtcgtgccagctgcattaatgaatcggccaacgcgcggggagaggcggtttgcgtattgggcgccagggtggtttttcttttcaccagtgagacgggcaacagctgattgcccttcaccgcctggccctgagagagttgcagcaagcggtccacgctggtttgccccagcaggcgaaaatcctgtttgatggtggttaacggcgggatataacatgagctgtcttcggtatcgtcgtatcccactaccgagatgtccgcaccaacgcgcagcccggactcggtaatggcgcgcattgcgcccagcgccatctgatcgttggcaaccagcatcgcagtgggaacgatgccctcattcagcatttgcatggtttgttgaaaaccggacatggcactccagtcgccttcccgttccgctatcggctgaatttgattgcgagtgagatatttatgccagccagccagacgcagacgcgccgagacagaacttaatgggcccgctaacagcgcgatttgctggtgacccaatgcgaccagatgctccacgcccagtcgcgtaccgtcttcatgggagaaaataatactgttgatgggtgtctggtcagagacatcaagaaataacgccggaacattagtgcaggcagcttccacagcaatggcatcctggtcatccagcggatagttaatgatcagcccactgacgcgttgcgcgagaagattgtgcaccgccgctttacaggcttcgacgccgcttcgttctaccatcgacaccaccacgctggcacccagttgatcggcgcgagatttaatcgccgcgacaatttgcgacggcgcgtgcagggccagactggaggtggcaacgccaatcagcaacgactgtttgcccgccagttgttgtgccacgcggttgggaatgtaattcagctccgccatcgccgcttccactttttcccgcgttttcgcagaaacgtggctggcctggttcaccacgcgggaaacggtctgataagagacaccggcatactctgcgacatcgtataacgttactggtttcacattcaccaccctgaattgactctcttccgggcgctatcatgccataccgcgaaaggttttgcgccattcgatggtgtccgggatctcgacgctctcccttatgcgactcctgcattaggaaattaatacgactcactata

SEQ ID NO: 13 - protein, 504 aa, Artificial Sequence
  Synthetic Construct
MEMNLLIDNWIPVRPRNGGKVQIINLQSLYCSRDQWRLSLPRDDMELAALALLVCIGQIIAPAKDDVEFRHRIMNPLTEDEFQQLIAPWIDMFYLNHAEHPFMQTKGVKANDVTPMEKLLAGVSGATNCAFVNQPGQGEALCGGCTAIALFNQANQAPGFGGGFKSGLRGGTPVTTFVRGIDLRSTVLLNVLTLPRLQKQFPNESHTENQPTWIKPIKSNESIPASSIGFVRGLFWQPAHIELCDPIGIGKCSCCGQESNLRYTGFLKEKFTFTVNGLWPHPHSPCLVTVKKGEVEEKFLAFTTSAPSWTQISRVVVDKIIQNENGNRVAAVVNQFRNIAPQSPLELIMGGYRNNQASILERRHDVLMFNQGWQQYGNVINEIVTVGLGYKTALRKALYTFAEGFKNKDFKGAGVSVHETAERHFYRQSELLIPDVLANVNFSQADEVIADLRDKLHQLCEMLFNQSVAPYAHHPKLISTLALARATLYKHLRELKPQGGPSNG

SEQ ID NO: 14 - DNA, 8166 bp, Artificial Sequence; identical to SEQ ID NO: 12
  (Cas8-Cas11-Cas7-bpNLS)+(Cas5-Cas6-bpNLS)/pRSFDuet-1
  CDS (1578)..(2060): Cas11

SEQ ID NO: 15 - protein, 160 aa, Artificial Sequence
  Synthetic Construct
MADEIDAMALYRAWQQLDNGSCAQIRRVSEPDELRDIPAFYRLVQPFGWENPRHQQALLRMVFCLSAGKNVIRHQDKKSEQTTGISLGRALANSGRINERRIFQLIRADRTADMVQLRRLLTHAEPVLDWPLMARMLTWWGKRERQQLLEDFVLTTNKNA

SEQ ID NO: 16 - DNA, 8166 bp, Artificial Sequence; identical to SEQ ID NO: 12
  (Cas8-Cas11-Cas7-bpNLS)+(Cas5-Cas6-bpNLS)/pRSFDuet-1
  CDS (2073)..(3218): Cas7-bpNLS

SEQ ID NO: 17 - protein, 381 aa, Artificial Sequence
  Synthetic Construct
MSNFINIHVLISHSPSCLNRDDMNMQKDAIFGGKRRVRISSQSLKRAMRKSGYYAQNIGESSLRTIHLAQLRDVLRQKLGERFDQKIIDKTLALLSGKSVDEAEKISADAVTPWVVGEIAWFCEQVAKAEADNLDDKKLLKVLKEDIAAIRVNLQQGVDIALSGRMATSGMMTELGKVDGAMSIAHAITTHQVDSDIDWFTAVDDLQEQGSAHLGTQEFSSGVFYRYANINLAQLQENLGGASREQALEIATHVVHMLATEVPGAKQRTYAAFNPADMVMVNFSDMPLSMANAFEKAVKAKDGFLQPSIQAFNQYWDRVANGYGLNGAAAQFSLSDVDPITAQVKQMPTLEQLKSWVRNNGEAKRTADGSEFESPKKKRKV

SEQ ID NO: 18 - DNA, 8166 bp, Artificial Sequence; identical to SEQ ID NO: 12
  (Cas8-Cas11-Cas7-bpNLS)+(Cas5-Cas6-bpNLS)/pRSFDuet-1
  CDS (3376)..(4050): Cas5

SEQ ID NO: 19 - protein, 224 aa, Artificial Sequence
  Synthetic Construct
MRSYLILRLAGPMQAWGQPTFEGTRPTGRFPTRSGLLGLLGACLGIQRDDTSSLQALSESVQFAVRCDELILDDRRVSVTGLRDYHTVLGAREDYRGLKSHETIQTWREYLCDASFTVALWLTPHATMVISELEKAVLKPRYTPYLGRRSCPLTHPLFLGTCQASDPQKALLNYEPVGGDIYSEESVTGHHLKFTARDEPMITLPRQFASREWYVIKGGMDVSQ

SEQ ID NO: 20 - DNA, 8166 bp, Artificial Sequence; identical to SEQ ID NO: 12
  (Cas8-Cas11-Cas7-bpNLS)+(Cas5-Cas6-bpNLS)/pRSFDuet-1
  CDS (4037)..(4690): Cas6-bpNLS

SEQ ID NO: 21 - protein, 217 aa, Artificial Sequence
  Synthetic Construct
MYLSKVIIARAWSRDLYQLHQGLWHLFPNRPDAARDFLFHVEKRNTPEGCHVLLQSAQMPVSTAVATVIKTKQVEFQLQVGVPLYFRLRANPIKTILDNQKRLDSKGNIKRCRVPLIKEAEQIAWLQRKLGNAARVEDVHPISERPQYFSGDGKSGKIQTVCFEGVLTINDAPALIDLVQQGIGPAKSMGCGLLSLAPLKRTADGSEFESPKKKRKV

SEQ ID NO: 22 - DNA, 4128 bp, Artificial Sequence
  EMX1-crRNA/pACYCDuet-1
  precursor_RNA (81)..(262): pre-crRNA
ggggaattgtgagcggataacaattcccctgtagaaataattttgtttaactttaataaggagatataccatggcatatgtggatgtgttgtttgtgtgatactataaagttggtagattgtgactggcttaaaaaatcattaattaataataggttatgtttagagtgttccccgcgccagcggggataaaccgcaggccaatggggaggacatcgatgtcacctcgtgttccccgcgccagcggggataaaccgttttttctcgaggcggccgcataatgcttaagtcgaacagaaagtaatcgtattgtacacggccgcataatcgaaattaatacgactcactataggggaattgtgagcggataacaattccccatcttagtatattagttaagtataagaaggagatatacatatggcagatctcaattggatatcggccggccacgcgatcgctgacgtcggtaccctcgagtctggtaaagaaaccgctgctgcgaaatttgaacgccagcacatggactcgtctactagcgcagcttaattaacctaggctgctgccaccgctgagcaataactagcataaccccttggggcctctaaacgggtcttgaggggttttttgctgaaacctcaggcatttgagaagcacacggtcacactgcttccggtagtcaataaaccggtaaaccagcaatagacataagcggctatttaacgaccctgccctgaaccgacgaccgggtcgaatttgctttcgaatttctgccattcatccgcttattatcacttattcaggcgtagcaccaggcgtttaagggcaccaataactgccttaaaaaaattacgccccgccctgccactcatcgcagtactgttgtaattcattaagcattctgccgacatggaagccatcacagacggcatgatgaacctgaatcgccagcggcatcagcaccttgtcgccttgcgtataatatttgcccatagtgaaaacgggggcgaagaagttgtccatattggccacgtttaaatcaaaactggtgaaactcacccagggattggctgagacgaaaaacatattctcaataaaccctttagggaaataggccaggttttcaccgtaacacgccacatcttgcgaatatatgtgtagaaactgccggaaatcgtcgtggtattcactccagagcgatgaaaacgtttcagtttgctcatggaaaacggtgtaacaagggtgaacactatcccatatcaccagctcaccgtctttcattgccatacggaactccggatgagcattcatcaggcgggcaagaatgtgaataaaggccggataaaacttgtgcttatttttctttacggtctttaaaaaggccgtaatatccagctgaacggtctggttataggtacattgagcaactgactgaaatgcctcaaaatgttctttacgatgccattgggatatatcaacggtggtatatccagtgatttttttctccattttagcttccttagctcctgaaaatctcgataactcaaaaaatacgcccggtagtgatcttatttcattatggtgaaagttggaacctcttacgtgccgatcaacgtctcattttcgccaaaagttggcccagggcttcccggtatcaacagggacaccaggatttatttattctgcgaagtgatcttccgtcacaggtatttattcggcgcaaagtgcgtcgggtgatgctgccaacttactgatttagtgtatgatggtgtttttgaggtgctccagtggcttctgtttctatcagctgtccctcctgttcagctactgacggggtggtgcgtaacggcaaaagcaccgccggacatcagcgctagcggagtgtatactggcttactatgttggcactgatgagggtgtcagtgaagtgcttcatgtggcaggagaaaaaaggctgcaccggtgcgtcagcagaatatgtgatacaggatatattccgcttcctcgctcactgactcgctacgctcggtcgttcgactgcggcgagcggaaatggcttacgaacggggcggagatttcctggaagatgccaggaagatacttaacagggaagtgagagggccgcggcaaagccgtttttccataggctccgcccccctgacaagcatcacgaaatctgacgctcaaatcagtggtggcgaaacccgacaggactataaagataccaggcgtttcccctggcggctccctcgtgcgctctcctgttcctgcctttcggtttaccggtgtcattccgctgttatggccgcgtttgtctcattccacgcctgacactcagttccgggtaggcagttcgctccaagctggactgtatgcacgaaccccccgttcagtccgaccgctgcgccttatccggtaactatcgtcttgagtccaacccggaaagacatgcaaaagcaccactggcagcagccactggtaattgatttagaggagttagtcttgaagtcatgcgccggttaaggctaaactgaaaggacaagttttggtgactgcgctcctccaagccagttacctcggttcaaagagttggtagctcagagaaccttcgaaaaaccgccctgcaaggcggttttttcgttttcagagcaagagattacgcgcagaccaaaacgatctcaagaagatcatcttattaatcagataaaatatttctagatttcagtgcaatttatctcttcaaatgtagcacctgaagtcagccccatacgatataagttgtaattctcatgttagtcatgccccgcgcccaccggaaggagctgactgggttgaaggctctcaagggcatcggtcgagatcccggtgcctaatgagtgagctaacttacattaattgcgttgcgctcactgcccgctttccagtcgggaaacctgtcgtgccagctgcattaatgaatcggccaacgcgcggggagaggcggtttgcgtattgggcgccagggtggtttttcttttcaccagtgagacgggcaacagctgattgcccttcaccgcctggccctgagagagttgcagcaagcggtccacgctggtttgccccagcaggcgaaaatcctgtttgatggtggttaacggcgggatataacatgagctgtcttcggtatcgtcgtatcccactaccgagatgtccgcaccaacgcgcagcccggactcggtaatggcgcgcattgcgcccagcgccatctgatcgttggcaaccagcatcgcagtgggaacgatgccctcattcagcatttgcatggtttgttgaaaaccggacatggcactccagtcgccttcccgttccgctatcggctgaatttgattgcgagtgagatatttatgccagccagccagacgcagacgcgccgagacagaacttaatgggcccgctaacagcgcgatttgctggtgacccaatgcgaccagatgctccacgcccagtcgcgtaccgtcttcatgggagaaaataatactgttgatgggtgtctggtcagagacatcaagaaataacgccggaacattagtgcaggcagcttccacagcaatggcatcctggtcatccagcggatagttaatgatcagcccactgacgcgttgcgcgagaagattgtgcaccgccgctttacaggcttcgacgccgcttcgttctaccatcgacaccaccacgctggcacccagttgatcggcgcgagatttaatcgccgcgacaatttgcgacggcgcgtgcagggccagactggaggtggcaacgccaatcagcaacgactgtttgcccgccagttgttgtgccacgcggttgggaatgtaattcagctccgccatcgccgcttccactttttcccgcgttttcgcagaaacgtggctggcctggttcaccacgcgggaaacggtctgataagagacaccggcatactctgcgacatcgtataacgttactggtttcacattcaccaccctgaattgactctcttccgggcgctatcatgccataccgcgaaaggttttgcgccattcgatggtgtccgggatctcgacgctctcccttatgcgactcctgcattaggaaattaatacgactcactata

SEQ ID NO: 23 - DNA, 4128 bp, Artificial Sequence
  Tyr-crRNA/pACYCDuet-1
  precursor_RNA (81)..(262): pre-crRNA
ggggaattgtgagcggataacaattcccctgtagaaataattttgtttaactttaataaggagatataccatggcatatgtggatgtgttgtttgtgtgatactataaagttggtagattgtgactggcttaaaaaatcattaattaataataggttatgtttagagtgttccccgcgccagcggggataaaccgggacacactgcttgggggctctgaaatatggagtgttccccgcgccagcggggataaaccgttttttctcgaggcggccgcataatgcttaagtcgaacagaaagtaatcgtattgtacacggccgcataatcgaaattaatacgactcactataggggaattgtgagcggataacaattccccatcttagtatattagttaagtataagaaggagatatacatatggcagatctcaattggatatcggccggccacgcgatcgctgacgtcggtaccctcgagtctggtaaagaaaccgctgctgcgaaatttgaacgccagcacatggactcgtctactagcgcagcttaattaacctaggctgctgccaccgctgagcaataactagcataaccccttggggcctctaaacgggtcttgaggggttttttgctgaaacctcaggcatttgagaagcacacggtcacactgcttccggtagtcaataaaccggtaaaccagcaatagacataagcggctatttaacgaccctgccctgaaccgacgaccgggtcgaatttgctttcgaatttctgccattcatccgcttattatcacttattcaggcgtagcaccaggcgtttaagggcaccaataactgccttaaaaaaattacgccccgccctgccactcatcgcagtactgttgtaattcattaagcattctgccgacatggaagccatcacagacggcatgatgaacctgaatcgccagcggcatcagcaccttgtcgccttgcgtataatatttgcccatagtgaaaacgggggcgaagaagttgtccatattggccacgtttaaatcaaaactggtgaaactcacccagggattggctgagacgaaaaacatattctcaataaaccctttagggaaataggccaggttttcaccgtaacacgccacatcttgcgaatatatgtgtagaaactgccggaaatcgtcgtggtattcactccagagcgatgaaaacgtttcagtttgctcatggaaaacggtgtaacaagggtgaacactatcccatatcaccagctcaccgtctttcattgccatacggaactccggatgagcattcatcaggcgggcaagaatgtgaataaaggccggataaaacttgtgcttatttttctttacggtctttaaaaaggccgtaatatccagctgaacggtctggttataggtacattgagcaactgactgaaatgcctcaaaatgttctttacgatgccattgggatatatcaacggtggtatatccagtgatttttttctccattttagcttccttagctcctgaaaatctcgataactcaaaaaatacgcccggtagtgatcttatttcattatggtgaaagttggaacctcttacgtgccgatcaacgtctcattttcgccaaaagttggcccagggcttcccggtatcaacagggacaccaggatttatttattctgcgaagtgatcttccgtcacaggtatttattcggcgcaaagtgcgtcgggtgatgctgccaacttactgatttagtgtatgatggtgtttttgaggtgctccagtggcttctgtttctatcagctgtccctcctgttcagctactgacggggtggtgcgtaacggcaaaagcaccgccggacatcagcgctagcggagtgtatactggcttactatgttggcactgatgagggtgtcagtgaagtgcttcatgtggcaggagaaaaaaggctgcaccggtgcgtcagcagaatatgtgatacaggatatattccgcttcctcgctcactgactcgctacgctcggtcgttcgactgcggcgagcggaaatggcttacgaacggggcggagatttcctggaagatgccaggaagatacttaacagggaagtgagagggccgcggcaaagccgtttttccataggctccgcccccctgacaagcatcacgaaatctgacgctcaaatcagtggtggcgaaacccgacaggactataaagataccaggcgtttcccctggcggctccctcgtgcgctctcctgttcctgcctttcggtttaccggtgtcattccgctgttatggccgcgtttgtctcattccacgcctgacactcagttccgggtaggcagttcgctccaagctggactgtatgcacgaaccccccgttcagtccgaccgctgcgccttatccggtaactatcgtcttgagtccaacccggaaagacatgcaaaagcaccactggcagcagccactggtaattgatttagaggagttagtcttgaagtcatgcgccggttaaggctaaactgaaaggacaagttttggtgactgcgctcctccaagccagttacctcggttcaaagagttggtagctcagagaaccttcgaaaaaccgccctgcaaggcggttttttcgttttcagagcaagagattacgcgcagaccaaaacgatctcaagaagatcatcttattaatcagataaaatatttctagatttcagtgcaatttatctcttcaaatgtagcacctgaagtcagccccatacgatataagttgtaattctcatgttagtcatgccccgcgcccaccggaaggagctgactgggttgaaggctctcaagggcatcggtcgagatcccggtgcctaatgagtgagctaacttacattaattgcgttgcgctcactgcccgctttccagtcgggaaacctgtcgtgccagctgcattaatgaatcggccaacgcgcggggagaggcggtttgcgtattgggcgccagggtggtttttcttttcaccagtgagacgggcaacagctgattgcccttcaccgcctggccctgagagagttgcagcaagcggtccacgctggtttgccccagcaggcgaaaatcctgtttgatggtggttaacggcgggatataacatgagctgtcttcggtatcgtcgtatcccactaccgagatgtccgcaccaacgcgcagcccggactcggtaatggcgcgcattgcgcccagcgccatctgatcgttggcaaccagcatcgcagtgggaacgatgccctcattcagcatttgcatggtttgttgaaaaccggacatggcactccagtcgccttcccgttccgctatcggctgaatttgattgcgagtgagatatttatgccagccagccagacgcagacgcgccgagacagaacttaatgggcccgctaacagcgcgatttgctggtgacccaatgcgaccagatgctccacgcccagtcgcgtaccgtcttcatgggagaaaataatactgttgatgggtgtctggtcagagacatcaagaaataacgccggaacattagtgcaggcagcttccacagcaatggcatcctggtcatccagcggatagttaatgatcagcccactgacgcgttgcgcgagaagattgtgcaccgccgctttacaggcttcgacgccgcttcgttctaccatcgacaccaccacgctggcacccagttgatcggcgcgagatttaatcgccgcgacaatttgcgacggcgcgtgcagggccagactggaggtggcaacgccaatcagcaacgactgtttgcccgccagttgttgtgccacgcggttgggaatgtaattcagctccgccatcgccgcttccactttttcccgcgttttcgcagaaacgtggctggcctggttcaccacgcgggaaacggtctgataagagacaccggcatactctgcgacatcgtataacgttactggtttcacattcaccaccctgaattgactctcttccgggcgctatcatgccataccgcgaaaggttttgcgccattcgatggtgtccgggatctcgacgctctcccttatgcgactcctgcattaggaaattaatacgactcactata

SEQ ID NO: 24 - DNA, 4128 bp, Artificial Sequence
  GFP-crRNA/pACYCDuet-1
  precursor_RNA (81)..(262): pre-crRNA
ggggaattgtgagcggataacaattcccctgtagaaataattttgtttaactttaataaggagatataccatggcatatgtggatgtgttgtttgtgtgatactataaagttggtagattgtgactggcttaaaaaatcattaattaataataggttatgtttagagtgttccccgcgccagcggggataaaccgatccgccacaacatcgaggacggcagcgtgcagtgttccccgcgccagcggggataaaccgttttttctcgaggcggccgcataatgcttaagtcgaacagaaagtaatcgtattgtacacggccgcataatcgaaattaatacgactcactataggggaattgtgagcggataacaattccccatcttagtatattagttaagtataagaaggagatatacatatggcagatctcaattggatatcggccggccacgcgatcgctgacgtcggtaccctcgagtctggtaaagaaaccgctgctgcgaaatttgaacgccagcacatggactcgtctactagcgcagcttaattaacctaggctgctgccaccgctgagcaataactagcataaccccttggggcctctaaacgggtcttgaggggttttttgctgaaacctcaggcatttgagaagcacacggtcacactgcttccggtagtcaataaaccggtaaaccagcaatagacataagcggctatttaacgaccctgccctgaaccgacgaccgggtcgaatttgctttcgaatttctgccattcatccgcttattatcacttattcaggcgtagcaccaggcgtttaagggcaccaataactgccttaaaaaaattacgccccgccctgccactcatcgcagtactgttgtaattcattaagcattctgccgacatggaagccatcacagacggcatgatgaacctgaatcgccagcggcatcagcaccttgtcgccttgcgtataatatttgcccatagtgaaaacgggggcgaagaagttgtccatattggccacgtttaaatcaaaactggtgaaactcacccagggattggctgagacgaaaaacatattctcaataaaccctttagggaaataggccaggttttcaccgtaacacgccacatcttgcgaatatatgtgtagaaactgccggaaatcgtcgtggtattcactccagagcgatgaaaacgtttcagtttgctcatggaaaacggtgtaacaagggtgaacactatcccatatcaccagctcaccgtctttcattgccatacggaactccggatgagcattcatcaggcgggcaagaatgtgaataaaggccggataaaacttgtgcttatttttctttacggtctttaaaaaggccgtaatatccagctgaacggtctggttataggtacattgagcaactgactgaaatgcctcaaaatgttctttacgatgccattgggatatatcaacggtggtatatccagtgatttttttctccattttagcttccttagctcctgaaaatctcgataactcaaaaaatacgcccggtagtgatcttatttcattatggtgaaagttggaacctcttacgtgccgatcaacgtctcattttcgccaaaagttggcccagggcttcccggtatcaacagggacaccaggatttatttattctgcgaagtgatcttccgtcacaggtatttattcggcgcaaagtgcgtcgggtgatgctgccaacttactgatttagtgtatgatggtgtttttgaggtgctccagtggcttctgtttctatcagctgtccctcctgttcagctactgacggggtggtgcgtaacggcaaaagcaccgccggacatcagcgctagcggagtgtatactggcttactatgttggcactgatgagggtgtcagtgaagtgcttcatgtggcaggagaaaaaaggctgcaccggtgcgtcagcagaatatgtgatacaggatatattccgcttcctcgctcactgactcgctacgctcggtcgttcgactgcggcgagcggaaatggcttacgaacggggcggagatttcctggaagatgccaggaagatacttaacagggaagtgagagggccgcggcaaagccgtttttccataggctccgcccccctgacaagcatcacgaaatctgacgctcaaatcagtggtggcgaaacccgacaggactataaagataccaggcgtttcccctggcggctccctcgtgcgctctcctgttcctgcctttcggtttaccggtgtcattccgctgttatggccgcgtttgtctcattccacgcctgacactcagttccgggtaggcagttcgctccaagctggactgtatgcacgaaccccccgttcagtccgaccgctgcgccttatccggtaactatcgtcttgagtccaacccggaaagacatgcaaaagcaccactggcagcagccactggtaattgatttagaggagttagtcttgaagtcatgcgccggttaaggctaaactgaaaggacaagttttggtgactgcgctcctccaagccagttacctcggttcaaagagttggtagctcagagaaccttcgaaaaaccgccctgcaaggcggttttttcgttttcagagcaagagattacgcgcagaccaaaacgatctcaagaagatcatcttattaatcagataaaatatttctagatttcagtgcaatttatctcttcaaatgtagcacctgaagtcagccccatacgatataagttgtaattctcatgttagtcatgccccgcgcccaccggaaggagctgactgggttgaaggctctcaagggcatcggtcgagatcccggtgcctaatgagtgagctaacttacattaattgcgttgcgctcactgcccgctttccagtcgggaaacctgtcgtgccagctgcattaatgaatcggccaacgcgcggggagaggcggtttgcgtattgggcgccagggtggtttttcttttcaccagtgagacgggcaacagctgattgcccttcaccgcctggccctgagagagttgcagcaagcggtccacgctggtttgccccagcaggcgaaaatcctgtttgatggtggttaacggcgggatataacatgagctgtcttcggtatcgtcgtatcccactaccgagatgtccgcaccaacgcgcagcccggactcggtaatggcgcgcattgcgcccagcgccatctgatcgttggcaaccagcatcgcagtgggaacgatgccctcattcagcatttgcatggtttgttgaaaaccggacatggcactccagtcgccttcccgttccgctatcggctgaatttgattgcgagtgagatatttatgccagccagccagacgcagacgcgccgagacagaacttaatgggcccgctaacagcgcgatttgctggtgacccaatgcgaccagatgctccacgcccagtcgcgtaccgtcttcatgggagaaaataatactgttgatgggtgtctggtcagagacatcaagaaataacgccggaacattagtgcaggcagcttccacagcaatggcatcctggtcatccagcggatagttaatgatcagcccactgacgcgttgcgcgagaagattgtgcaccgccgctttacaggcttcgacgccgcttcgttctaccatcgacaccaccacgctggcacccagttgatcggcgcgagatttaatcgccgcgacaatttgcgacggcgcgtgcagggccagactggaggtggcaacgccaatcagcaacgactgtttgcccgccagttgttgtgccacgcggttgggaatgtaattcagctccgccatcgccgcttccactttttcccgcgttttcgcagaaacgtggctggcctggttcaccacgcgggaaacggtctgataagagacaccggcatactctgcgacatcgtataacgttactggtttcacattcaccaccctgaattgactctcttccgggcgctatcatgccataccgcgaaaggttttgcgccattcgatggtgtccgggatctcgacgctctcccttatgcgactcctgcattaggaaattaatacgactcactata